European Patent Application EP 4 710 942 A1, published March 18, 2026. Title: 一种高效靶向胶质瘤起始细胞的siRNA共递药体系的制备及应用. Applicant: 天津键凯科技有限公司. The sequence listing filed with the application follows.

SEQUENCE LISTING (9 sequences)

SEQ ID NO: 1 - RNA, 21 nt, synthetic construct
  source 1..21: mol_type = other RNA
  modified_base 20..21: mod_base = OTHER; note = thymine
tgccaaatgcctgccagaatt

SEQ ID NO: 2 - RNA, 21 nt, synthetic construct
  source 1..21: mol_type = other RNA
  modified_base 20..21: mod_base = OTHER; note = thymine
ttctggcaggcatttggcatt

SEQ ID NO: 3 - protein, 7 aa, synthetic construct
  SITE 1: note = D-serine
  SITE 2: note = D-asparagine
  SITE 3: note = D-threonine
  SITE 4: note = D-arginine
  SITE 5: note = D-valine
  SITE 6: note = D-alanine
  SITE 7: note = D-proline
SNTRVAP

SEQ ID NO: 4 - RNA, 21 nt, synthetic construct
  source 1..21: mol_type = other RNA
  modified_base 20..21: mod_base = OTHER; note = thymine
ttctccgaacgtgtcacgttt

SEQ ID NO: 5 - RNA, 21 nt, synthetic construct
  source 1..21: mol_type = other RNA
  modified_base 20..21: mod_base = OTHER; note = thymine
acgtgacacgttcggagaatt

SEQ ID NO: 6 - DNA, 19 bp, synthetic construct
  source 1..19: mol_type = other DNA
cagaggcgtggcagactat

SEQ ID NO: 7 - DNA, 20 bp, synthetic construct
  source 1..20: mol_type = other DNA
ggcacttgtactccgtcagc

SEQ ID NO: 8 - DNA, 19 bp, synthetic construct
  source 1..19: mol_type = other DNA
tggcacccagcacaatgaa

SEQ ID NO: 9 - DNA, 21 bp, synthetic construct
  source 1..21: mol_type = other DNA
ctaagtcatagtccgcctaga